European Patent Application EP 4 768 502 A1, published July 1, 2026. Title: ANTI-CORONAVIRUS ANTIBODY. Applicant: CEVA SANTE ANIMALE. The sequence listing filed with the application follows.

SEQUENCE LISTING (5 sequences)

SEQ ID NO: 1 - protein, 5 aa, synthetic construct
FVAMA

SEQ ID NO: 2 - protein, 17 aa, synthetic construct
RISSTGTVTNYADSVKG

SEQ ID NO: 3 - protein, 7 aa, synthetic construct
VPGNLLP

SEQ ID NO: 4 - protein, 116 aa, synthetic construct
EVQLVESGGGLVQAGGSLRLSCAASGSLLSFVAMAWYRQVPGKEREVVARISSTGTVTNYADSVKGRFTISRDNAKKTLDLQMNSLKPEDTAVYYCNRVPGNLLPWGQGTQVTVSS

SEQ ID NO: 5 - protein, 242 aa, unidentified
EVQLVESGGGLVQAGGSLRLSCAASGSLLSFVAMAWYRQVPGKEREVVARISSTGTVTNYADSVKGRFTISRDNAKKTLDLQMNSLKPEDTAVYYCNRVPGNLLPWGQGTQVTVSSGSGSGSGSGSEVQLVESGGGLVQAGGSLRLSCAASGSLLSFVAMAWYRQVPGKEREVVARISSTGTVTNYADSVKGRFTISRDNAKKTLDLQMNSLKPEDTAVYYCNRVPGNLLPWGQGTQVTVSS